European Patent Specification EP 3 279 214 B1, published October 9, 2024. Title: Method for the production of immunoglobulin single variable domains. Applicant: Ablynx N.V. The sequence listing filed with the application follows.

SEQUENCE LISTING (5 sequences)

SEQ ID NO: 1 - protein, 245 aa, Artificial Sequence
  Nanobody sequence
EVQLVESGGGLVQPGGSLRLSCAASGSVFKINVMAWYRQAPGKGRELVAGIISGGSTSYADSVKGRFTISRDNAKNTLYLQMNSLRPEDTAVYYCAFITTESDYDLGRRYWGQGTLVTVSSGGGGSGGGSEVQLVESGGGLVQPGNSLRLSCAASGFTFSSFGMSWVRQAPGKGLEWVSSISGSGSDTLYADSVKGRFTISRDNAKTTLYLQMNSLRPEDTAVYYCTIGGSLSRSSQGTLVTVSS

SEQ ID NO: 2 - protein, 120 aa, Artificial Sequence
  Nanobody sequence
EVQLVESGGGFVQAGGSLRLSCIASGDNFSINRMGWYRQALGKQRELVAIITNHGSTNYADAVKGRFTISRDYAKNTVYLQMNGLKPDDTAVYYCNAYISEVGTWRDDYWGQGIQVTVSS

SEQ ID NO: 3 - protein, 270 aa, Artificial Sequence
  Nanobody sequence
EVQLVESGGGLVQPGGSLRLSCAASGFTFSSYAMSWVRQAPGKGLEWVSGIKSSGDSTRYAGSVKGRFTISRDNAKNTLYLQMNSLRPEDTAVYYCAKSRVSRTGLYTYDNRGQGTLVTVSSGGGGSGGGGSGGGGSGGGGSEVQLVESGGGLVQPGGSLRLSCAASGRTFNNYAMGWFRQAPGKEREFVAAITRSGVRSGVSAIYGDSVKDRFTISRDNAKNTLYLQMNSLRPEDTAVYYCAASAIGSGALRRFEYDYSGQGTLVTVSS

SEQ ID NO: 4 - protein, 408 aa, Artificial Sequence
  Nanobody sequence
DVQLVESGGGLVQAGGSLSISCAASGGSLSNYVLGWFRQAPGKEREFVAAINWRGDITIGPPNVEGRFTISRDNAKNTGYLQMNSLAPDDTAVYYCGAGTPLNPGAYIYDWSYDYWGRGTQVTVSSGGGGSGGGGSGGGGSEVQLVESGGGLVQAGGSLSISCAASGGSLSNYVLGWFRQAPGKEREFVAAINWRGDITIGPPNVEGRFTISRDNAKNTGYLQMNSLAPDDTAVYYCGAGTPLNPGAYIYDWSYDYWGRGTQVTVSSGGGGSGGGGSGGGGSEVQLVESGGGLVQAGGSLSISCAASGGSLSNYVLGWFRQAPGKEREFVAAINWRGDITIGPPNVEGRFTISRDNAKNTGYLQMNSLAPDDTAVYYCGAGTPLNPGAYIYDWSYDYWGRGTQVTVSS

SEQ ID NO: 5 - protein, 367 aa, Artificial Sequence
  Nanobody sequence
DVQLVESGGGLVQPGGSLRLSCAASRSIGRLDRMGWYRHRPGEPRELVATITGGSSINYGDSVKGRFTISIDNSKNTVYLQMNSLRPEDTAVYYCNFNKYVTSRDTWGQGTLVTVSSGGGGSGGGSEVQLVESGGGLVQPGNSLRLSCAASGFTFSSFGMSWVRQAPGKGLEWVSSISGSGSDTLYADSVKGRFTISRDNAKTTLYLQMNSLRPEDTAVYYCTIGGSLSRSSQGTLVTVSSGGGGSGGGSEVQLVESGGGLVQPGGSLRLSCAASRSIGRLDRMGWYRHRPGEPRELVATITGGSSINYGDSVKGRFTISIDNSKNTVYLQMNSLRPEDTAVYYCNFNKYVTSRDTWGQGTLVTVSS